European Patent Application EP 4 455 285 A2, published October 30, 2024. Title: NUCLEIC ACID, COMPOSITION AND CONJUGATE COMPRISING THE SAME, AND PREPARATION METHOD AND USE THEREOF. Applicant: Suzhou Ribo Life Science Co., Ltd. Application EP. The sequence listing filed with the application follows.

SEQUENCE LISTING (156 sequences)

SEQ ID NO: 1 - RNA, 19 nt, synthetic construct
  misc_feature 19: note = n selected from A, U, G, or C
  source 1..19: mol_type = other RNA
ccttgaggcatacttcaan

SEQ ID NO: 2 - RNA, 19 nt, synthetic construct
  misc_feature 1: note = n selected from A, U, G, or C
  source 1..19: mol_type = other RNA
nttgaagtatgcctcaagg

SEQ ID NO: 3 - RNA, 21 nt, synthetic construct
  misc_feature 1: note = n selected from A, U, G, or C
  source 1..21: mol_type = other RNA
nttgaagtatgcctcaaggtt

SEQ ID NO: 4 - RNA, 21 nt, synthetic construct
  misc_feature 1: note = n selected from A, U, G, or C
  source 1..21: mol_type = other RNA
nttgaagtatgcctcaaggtc

SEQ ID NO: 5 - RNA, 19 nt, synthetic construct
  source 1..19: mol_type = other RNA
ccttgaggcatacttcaaa

SEQ ID NO: 6 - RNA, 21 nt, synthetic construct
  source 1..21: mol_type = other RNA
tttgaagtatgcctcaaggtt

SEQ ID NO: 7 - RNA, 21 nt, synthetic construct
  source 1..21: mol_type = other RNA
gaccttgaggcatacttcaaa

SEQ ID NO: 8 - RNA, 23 nt, synthetic construct
  source 1..23: mol_type = other RNA
tttgaagtatgcctcaaggtcgg

SEQ ID NO: 9 - RNA, 19 nt, synthetic construct
  source 1..19: mol_type = other RNA
ccttgaggcatacttcaaa

SEQ ID NO: 10 - RNA, 21 nt, synthetic construct
  source 1..21: mol_type = other RNA
tttgaagtatgcctcaaggtt

SEQ ID NO: 11 - RNA, 19 nt, synthetic construct
  source 1..19: mol_type = other RNA
ccttgaggcatacttcaaa

SEQ ID NO: 12 - RNA, 21 nt, synthetic construct
  source 1..21: mol_type = other RNA
tttgaagtatgcctcaaggtt

SEQ ID NO: 13 - RNA, 21 nt, synthetic construct
  source 1..21: mol_type = other RNA
gaccttgaggcatacttcaaa

SEQ ID NO: 14 - RNA, 23 nt, synthetic construct
  source 1..23: mol_type = other RNA
tttgaagtatgcctcaaggtcgg

SEQ ID NO: 15 - RNA, 21 nt, synthetic construct
  source 1..21: mol_type = other RNA
gaccttgaggcatacttcaaa

SEQ ID NO: 16 - RNA, 23 nt, synthetic construct
  source 1..23: mol_type = other RNA
tttgaagtatgcctcaaggtcgg

SEQ ID NO: 17 - RNA, 19 nt, synthetic construct
  source 1..19: mol_type = other RNA
ccttgaggcatacttcaaa

SEQ ID NO: 18 - RNA, 21 nt, synthetic construct
  source 1..21: mol_type = other RNA
tttgaagtatgcctcaaggtt

SEQ ID NO: 19 - RNA, 19 nt, synthetic construct
  source 1..19: mol_type = other RNA
ccttgaggcatacttcaaa

SEQ ID NO: 20 - RNA, 21 nt, synthetic construct
  source 1..21: mol_type = other RNA
tttgaagtatgcctcaaggtt

SEQ ID NO: 21 - RNA, 21 nt, synthetic construct
  source 1..21: mol_type = other RNA
gaccttgaggcatacttcaaa

SEQ ID NO: 22 - RNA, 23 nt, synthetic construct
  source 1..23: mol_type = other RNA
tttgaagtatgcctcaaggtcgg

SEQ ID NO: 23 - RNA, 21 nt, synthetic construct
  source 1..21: mol_type = other RNA
gaccttgaggcatacttcaaa

SEQ ID NO: 24 - RNA, 23 nt, synthetic construct
  source 1..23: mol_type = other RNA
tttgaagtatgcctcaaggtcgg

SEQ ID NO: 25 - RNA, 19 nt, synthetic construct
  source 1..19: mol_type = other RNA
ccttgaggcatacttcaaa

SEQ ID NO: 26 - RNA, 21 nt, synthetic construct
  source 1..21: mol_type = other RNA
tttgaagtatgcctcaaggtt

SEQ ID NO: 27 - RNA, 19 nt, synthetic construct
  source 1..19: mol_type = other RNA
ccttgaggcatacttcaaa

SEQ ID NO: 28 - RNA, 21 nt, synthetic construct
  source 1..21: mol_type = other RNA
tttgaagtatgcctcaaggtt

SEQ ID NO: 29 - RNA, 21 nt, synthetic construct
  source 1..21: mol_type = other RNA
gaccttgaggcatacttcaaa

SEQ ID NO: 30 - RNA, 23 nt, synthetic construct
  source 1..23: mol_type = other RNA
tttgaagtatgcctcaaggtcgg

SEQ ID NO: 31 - RNA, 21 nt, synthetic construct
  source 1..21: mol_type = other RNA
gaccttgaggcatacttcaaa

SEQ ID NO: 32 - RNA, 23 nt, synthetic construct
  source 1..23: mol_type = other RNA
tttgaagtatgcctcaaggtcgg

SEQ ID NO: 33 - RNA, 19 nt, synthetic construct
  source 1..19: mol_type = other RNA
ccttgaggcatacttcaaa

SEQ ID NO: 34 - RNA, 21 nt, synthetic construct
  source 1..21: mol_type = other RNA
tttgaagtatgcctcaaggtt

SEQ ID NO: 35 - RNA, 19 nt, synthetic construct
  source 1..19: mol_type = other RNA
ccttgaggcatacttcaaa

SEQ ID NO: 36 - RNA, 21 nt, synthetic construct
  source 1..21: mol_type = other RNA
tttgaagtatgcctcaaggtt

SEQ ID NO: 37 - RNA, 21 nt, synthetic construct
  source 1..21: mol_type = other RNA
gaccttgaggcatacttcaaa

SEQ ID NO: 38 - RNA, 23 nt, synthetic construct
  source 1..23: mol_type = other RNA
tttgaagtatgcctcaaggtcgg

SEQ ID NO: 39 - RNA, 21 nt, synthetic construct
  source 1..21: mol_type = other RNA
gaccttgaggcatacttcaaa

SEQ ID NO: 40 - RNA, 23 nt, synthetic construct
  source 1..23: mol_type = other RNA
tttgaagtatgcctcaaggtcgg

SEQ ID NO: 41 - RNA, 19 nt, synthetic construct
  source 1..19: mol_type = other RNA
ccttgaggcatacttcaaa

SEQ ID NO: 42 - RNA, 21 nt, synthetic construct
  source 1..21: mol_type = other RNA
tttgaagtatgcctcaaggtt

SEQ ID NO: 43 - RNA, 19 nt, synthetic construct
  source 1..19: mol_type = other RNA
ccttgaggcatacttcaaa

SEQ ID NO: 44 - RNA, 21 nt, synthetic construct
  source 1..21: mol_type = other RNA
tttgaagtatgcctcaaggtt

SEQ ID NO: 45 - RNA, 19 nt, synthetic construct
  source 1..19: mol_type = other RNA
ccttgaggcatacttcaaa

SEQ ID NO: 46 - RNA, 21 nt, synthetic construct
  modified_base 1: mod_base = OTHER; note = thymine
  source 1..21: mol_type = other RNA
tttgaagtatgcctcaaggtt

SEQ ID NO: 47 - RNA, 19 nt, synthetic construct
  source 1..19: mol_type = other RNA
ccttgaggcatacttcaaa

SEQ ID NO: 48 - RNA, 21 nt, synthetic construct
  source 1..21: mol_type = other RNA
tttgaagtatgcctcaaggtt

SEQ ID NO: 49 - RNA, 19 nt, synthetic construct
  source 1..19: mol_type = other RNA
ccttgaggcatacttcaaa

SEQ ID NO: 50 - RNA, 21 nt, synthetic construct
  source 1..21: mol_type = other RNA
tttgaagtatgcctcaaggtt

SEQ ID NO: 51 - RNA, 19 nt, synthetic construct
  source 1..19: mol_type = other RNA
ccttgaggcatacttcaaa

SEQ ID NO: 52 - RNA, 21 nt, synthetic construct
  source 1..21: mol_type = other RNA
tttgaagtatgcctcaaggtt

SEQ ID NO: 53 - RNA, 21 nt, synthetic construct
  source 1..21: mol_type = other RNA
gaccttgaggcatacttcaaa

SEQ ID NO: 54 - RNA, 23 nt, synthetic construct
  source 1..23: mol_type = other RNA
tttgaagtatgcctcaaggtcgg

SEQ ID NO: 55 - RNA, 19 nt, synthetic construct
  source 1..19: mol_type = other RNA
ccttgaggcatacttcaaa

SEQ ID NO: 56 - RNA, 21 nt, synthetic construct
  source 1..21: mol_type = other RNA
tttgaagtatgcctcaaggtt

SEQ ID NO: 57 - RNA, 19 nt, synthetic construct
  source 1..19: mol_type = other RNA
ccttgaggcatacttcaaa

SEQ ID NO: 58 - RNA, 21 nt, synthetic construct
  source 1..21: mol_type = other RNA
tttgaagtatgcctcaaggtt

SEQ ID NO: 59 - RNA, 21 nt, synthetic construct
  source 1..21: mol_type = other RNA
gaccttgaggcatacttcaaa

SEQ ID NO: 60 - RNA, 23 nt, synthetic construct
  source 1..23: mol_type = other RNA
tttgaagtatgcctcaaggtcgg

SEQ ID NO: 61 - RNA, 21 nt, synthetic construct
  source 1..21: mol_type = other RNA
gaccttgaggcatacttcaaa

SEQ ID NO: 62 - RNA, 23 nt, synthetic construct
  source 1..23: mol_type = other RNA
tttgaagtatgcctcaaggtcgg

SEQ ID NO: 63 - RNA, 19 nt, synthetic construct
  source 1..19: mol_type = other RNA
ccttgaggcatacttcaaa

SEQ ID NO: 64 - RNA, 21 nt, synthetic construct
  source 1..21: mol_type = other RNA
tttgaagtatgcctcaaggtt

SEQ ID NO: 65 - RNA, 21 nt, synthetic construct
  source 1..21: mol_type = other RNA
gaccttgaggcatacttcaaa

SEQ ID NO: 66 - RNA, 23 nt, synthetic construct
  source 1..23: mol_type = other RNA
tttgaagtatgcctcaaggtcgg

SEQ ID NO: 67 - RNA, 19 nt, synthetic construct
  source 1..19: mol_type = other RNA
ccttgaggcatacttcaaa

SEQ ID NO: 68 - RNA, 21 nt, synthetic construct
  source 1..21: mol_type = other RNA
tttgaagtatgcctcaaggtt

SEQ ID NO: 69 - RNA, 19 nt, synthetic construct
  source 1..19: mol_type = other RNA
ccttgaggcatacttcaaa

SEQ ID NO: 70 - RNA, 21 nt, synthetic construct
  source 1..21: mol_type = other RNA
tttgaagtatgcctcaaggtt

SEQ ID NO: 71 - RNA, 21 nt, synthetic construct
  source 1..21: mol_type = other RNA
gaccttgaggcatacttcaaa

SEQ ID NO: 72 - RNA, 23 nt, synthetic construct
  source 1..23: mol_type = other RNA
tttgaagtatgcctcaaggtcgg

SEQ ID NO: 73 - RNA, 21 nt, synthetic construct
  source 1..21: mol_type = other RNA
gaccttgaggcatacttcaaa

SEQ ID NO: 74 - RNA, 23 nt, synthetic construct
  source 1..23: mol_type = other RNA
tttgaagtatgcctcaaggtcgg

SEQ ID NO: 75 - RNA, 21 nt, synthetic construct
  source 1..21: mol_type = other RNA
gaccttgaggcatacttcaaa

SEQ ID NO: 76 - RNA, 23 nt, synthetic construct
  source 1..23: mol_type = other RNA
tttgaagtatgcctcaaggtcgg

SEQ ID NO: 77 - RNA, 19 nt, synthetic construct
  source 1..19: mol_type = other RNA
ccttgaggcatacttcaaa

SEQ ID NO: 78 - RNA, 21 nt, synthetic construct
  source 1..21: mol_type = other RNA
tttgaagtatgcctcaaggtt

SEQ ID NO: 79 - RNA, 19 nt, synthetic construct
  source 1..19: mol_type = other RNA
ccttgaggcatacttcaaa

SEQ ID NO: 80 - RNA, 21 nt, synthetic construct
  source 1..21: mol_type = other RNA
tttgaagtatgcctcaaggtt

SEQ ID NO: 81 - RNA, 21 nt, synthetic construct
  source 1..21: mol_type = other RNA
gaccttgaggcatacttcaaa

SEQ ID NO: 82 - RNA, 23 nt, synthetic construct
  source 1..23: mol_type = other RNA
tttgaagtatgcctcaaggtcgg

SEQ ID NO: 83 - RNA, 21 nt, synthetic construct
  source 1..21: mol_type = other RNA
gaccttgaggcatacttcaaa

SEQ ID NO: 84 - RNA, 23 nt, synthetic construct
  source 1..23: mol_type = other RNA
tttgaagtatgcctcaaggtcgg

SEQ ID NO: 85 - RNA, 21 nt, synthetic construct
  source 1..21: mol_type = other RNA
gaccttgaggcatacttcaaa

SEQ ID NO: 86 - RNA, 23 nt, synthetic construct
  source 1..23: mol_type = other RNA
tttgaagtatgcctcaaggtcgg

SEQ ID NO: 87 - RNA, 19 nt, synthetic construct
  source 1..19: mol_type = other RNA
ccttgaggcatacttcaaa

SEQ ID NO: 88 - RNA, 21 nt, synthetic construct
  source 1..21: mol_type = other RNA
tttgaagtatgcctcaaggtt

SEQ ID NO: 89 - RNA, 19 nt, synthetic construct
  source 1..19: mol_type = other RNA
ccttgaggcatacttcaaa

SEQ ID NO: 90 - RNA, 21 nt, synthetic construct
  source 1..21: mol_type = other RNA
tttgaagtatgcctcaaggtt

SEQ ID NO: 91 - RNA, 19 nt, synthetic construct
  source 1..19: mol_type = other RNA
ccttgaggcatacttcaaa

SEQ ID NO: 92 - RNA, 21 nt, synthetic construct
  source 1..21: mol_type = other RNA
tttgaagtatgcctcaaggtt

SEQ ID NO: 93 - RNA, 19 nt, synthetic construct
  source 1..19: mol_type = other RNA
ccttgaggcatacttcaaa

SEQ ID NO: 94 - RNA, 21 nt, synthetic construct
  source 1..21: mol_type = other RNA
tttgaagtatgcctcaaggtt

SEQ ID NO: 95 - RNA, 19 nt, synthetic construct
  source 1..19: mol_type = other RNA
ccttgaggcatacttcaaa

SEQ ID NO: 96 - RNA, 21 nt, synthetic construct
  source 1..21: mol_type = other RNA
tttgaagtatgcctcaaggtt

SEQ ID NO: 97 - RNA, 19 nt, synthetic construct
  source 1..19: mol_type = other RNA
ccttgaggcatacttcaaa

SEQ ID NO: 98 - RNA, 21 nt, synthetic construct
  source 1..21: mol_type = other RNA
tttgaagtatgcctcaaggtt

SEQ ID NO: 99 - RNA, 19 nt, synthetic construct
  source 1..19: mol_type = other RNA
ccttgaggcatacttcaaa

SEQ ID NO: 100 - RNA, 21 nt, synthetic construct
  source 1..21: mol_type = other RNA
tttgaagtatgcctcaaggtt

SEQ ID NO: 101 - RNA, 19 nt, synthetic construct
  source 1..19: mol_type = other RNA
ccttgaggcatacttcaaa

SEQ ID NO: 102 - RNA, 21 nt, synthetic construct
  source 1..21: mol_type = other RNA
tttgaagtatgcctcaaggtt

SEQ ID NO: 103 - RNA, 19 nt, synthetic construct
  source 1..19: mol_type = other RNA
ccttgaggcatacttcaaa

SEQ ID NO: 104 - RNA, 21 nt, synthetic construct
  source 1..21: mol_type = other RNA
tttgaagtatgcctcaaggtt

SEQ ID NO: 105 - RNA, 19 nt, synthetic construct
  source 1..19: mol_type = other RNA
ccttgaggcatacttcaaa

SEQ ID NO: 106 - RNA, 21 nt, synthetic construct
  source 1..21: mol_type = other RNA
tttgaagtatgcctcaaggtt

SEQ ID NO: 107 - RNA, 19 nt, synthetic construct
  source 1..19: mol_type = other RNA
ccttgaggcatacttcaaa

SEQ ID NO: 108 - RNA, 21 nt, synthetic construct
  source 1..21: mol_type = other RNA
tttgaagtatgcctcaaggtt

SEQ ID NO: 109 - RNA, 21 nt, synthetic construct
  source 1..21: mol_type = other RNA
gaccttgaggcatacttcaaa

SEQ ID NO: 110 - RNA, 23 nt, synthetic construct
  source 1..23: mol_type = other RNA
tttgaagtatgcctcaaggtcgg

SEQ ID NO: 111 - RNA, 21 nt, synthetic construct
  source 1..21: mol_type = other RNA
gaccttgaggcatacttcaaa

SEQ ID NO: 112 - RNA, 23 nt, synthetic construct
  source 1..23: mol_type = other RNA
tttgaagtatgcctcaaggtcgg

SEQ ID NO: 113 - RNA, 21 nt, synthetic construct
  source 1..21: mol_type = other RNA
gaccttgaggcatacttcaaa

SEQ ID NO: 114 - RNA, 23 nt, synthetic construct
  source 1..23: mol_type = other RNA
tttgaagtatgcctcaaggtcgg

SEQ ID NO: 115 - RNA, 21 nt, synthetic construct
  source 1..21: mol_type = other RNA
gaccttgaggcatacttcaaa

SEQ ID NO: 116 - RNA, 23 nt, synthetic construct
  source 1..23: mol_type = other RNA
tttgaagtatgcctcaaggtcgg

SEQ ID NO: 117 - RNA, 21 nt, synthetic construct
  source 1..21: mol_type = other RNA
gaccttgaggcatacttcaaa

SEQ ID NO: 118 - RNA, 23 nt, synthetic construct
  source 1..23: mol_type = other RNA
tttgaagtatgcctcaaggtcgg

SEQ ID NO: 119 - RNA, 21 nt, synthetic construct
  source 1..21: mol_type = other RNA
gaccttgaggcatacttcaaa

SEQ ID NO: 120 - RNA, 23 nt, synthetic construct
  source 1..23: mol_type = other RNA
tttgaagtatgcctcaaggtcgg

SEQ ID NO: 121 - RNA, 19 nt, synthetic construct
  source 1..19: mol_type = other RNA
ccttgaggcatacttcaaa

SEQ ID NO: 122 - RNA, 21 nt, synthetic construct
  source 1..21: mol_type = other RNA
tttgaagtatgcctcaaggtc

SEQ ID NO: 123 - RNA, 19 nt, synthetic construct
  source 1..19: mol_type = other RNA
ccttgaggcatacttcaaa

SEQ ID NO: 124 - RNA, 21 nt, synthetic construct
  source 1..21: mol_type = other RNA
tttgaagtatgcctcaaggtc

SEQ ID NO: 125 - RNA, 19 nt, synthetic construct
  source 1..19: mol_type = other RNA
ccttgaggcatacttcaaa

SEQ ID NO: 126 - RNA, 21 nt, synthetic construct
  source 1..21: mol_type = other RNA
tttgaagtatgcctcaaggtt

SEQ ID NO: 127 - RNA, 19 nt, synthetic construct
  source 1..19: mol_type = other RNA
ccttgaggcatacttcaaa

SEQ ID NO: 128 - RNA, 21 nt, synthetic construct
  source 1..21: mol_type = other RNA
tttgaagtatgcctcaaggtt

SEQ ID NO: 129 - RNA, 19 nt, synthetic construct
  source 1..19: mol_type = other RNA
ccttgaggcatacttcaaa

SEQ ID NO: 130 - RNA, 21 nt, synthetic construct
  source 1..21: mol_type = other RNA
tttgaagtatgcctcaaggtt

SEQ ID NO: 131 - RNA, 19 nt, synthetic construct
  source 1..19: mol_type = other RNA
ccttgaggcatacttcaaa

SEQ ID NO: 132 - RNA, 21 nt, synthetic construct
  source 1..21: mol_type = other RNA
tttgaagtatgcctcaaggtt

SEQ ID NO: 133 - RNA, 21 nt, synthetic construct
  source 1..21: mol_type = other RNA
gaccttgaggcatacttcaaa

SEQ ID NO: 134 - RNA, 23 nt, synthetic construct
  source 1..23: mol_type = other RNA
tttgaagtatgcctcaaggtcgg

SEQ ID NO: 135 - RNA, 19 nt, synthetic construct
  source 1..19: mol_type = other RNA
ccttgaggcatacttcaaa

SEQ ID NO: 136 - RNA, 21 nt, synthetic construct
  source 1..21: mol_type = other RNA
tttgaagtatgcctcaaggtt

SEQ ID NO: 137 - RNA, 21 nt, synthetic construct
  modified_base 20..21: mod_base = OTHER; note = thymine
  source 1..21: mol_type = other RNA
ccttgaggcatacttcaaatt

SEQ ID NO: 138 - RNA, 21 nt, synthetic construct
  modified_base 20..21: mod_base = OTHER; note = thymine
  source 1..21: mol_type = other RNA
tttgaagtatgcctcaaggtt

SEQ ID NO: 139 - RNA, 19 nt, synthetic construct
  source 1..19: mol_type = other RNA
ttctccgaacgtgtcacgt

SEQ ID NO: 140 - RNA, 21 nt, synthetic construct
  source 1..21: mol_type = other RNA
acgtgacacgttcggagaatt

SEQ ID NO: 141 - RNA, 19 nt, synthetic construct
  source 1..19: mol_type = other RNA
gtgtgcacttcgcttcaca

SEQ ID NO: 142 - RNA, 21 nt, synthetic construct
  source 1..21: mol_type = other RNA
tgtgaagcgaagtgcacactt

SEQ ID NO: 143 - RNA, 19 nt, synthetic construct
  source 1..19: mol_type = other RNA
ccttgaggcatacttcaaa

SEQ ID NO: 144 - RNA, 21 nt, synthetic construct
  source 1..21: mol_type = other RNA
tttgaagtatgcctcaaggtc

SEQ ID NO: 145 - RNA, 19 nt, synthetic construct
  source 1..19: mol_type = other RNA
ccttgaggcatacttcaaa

SEQ ID NO: 146 - RNA, 21 nt, synthetic construct
  source 1..21: mol_type = other RNA
tttgaagtatgcctcaaggtc

SEQ ID NO: 147 - RNA, 19 nt, synthetic construct
  source 1..19: mol_type = other RNA
ccttgaggcatacttcaaa

SEQ ID NO: 148 - RNA, 21 nt, synthetic construct
  source 1..21: mol_type = other RNA
tttgaagtatgcctcaaggtt

SEQ ID NO: 149 - RNA, 21 nt, synthetic construct
  modified_base 20..21: mod_base = OTHER; note = thymine
  source 1..21: mol_type = other RNA
ccttgaggcatacttcaaatt

SEQ ID NO: 150 - RNA, 21 nt, synthetic construct
  modified_base 20..21: mod_base = OTHER; note = thymine
  source 1..21: mol_type = other RNA
tttgaagtatgcctcaaggtt

SEQ ID NO: 151 - DNA, 20 bp, synthetic construct
  source 1..20: mol_type = other DNA
ccgtctgtgccttctcatct

SEQ ID NO: 152 - DNA, 20 bp, synthetic construct
  source 1..20: mol_type = other DNA
taatctcctcccccaactcc

SEQ ID NO: 153 - DNA, 24 bp, synthetic construct
  source 1..24: mol_type = other DNA
agcttctttgcagctccttcgttg

SEQ ID NO: 154 - DNA, 24 bp, synthetic construct
  source 1..24: mol_type = other DNA
ttctgacccattcccaccatcaca

SEQ ID NO: 155 - RNA, 19 nt, synthetic construct
  misc_feature 19: note = n is A
  source 1..19: mol_type = other RNA
ccttgaggcatacttcaan

SEQ ID NO: 156 - RNA, 19 nt, synthetic construct
  misc_feature 1: note = n is U
  source 1..19: mol_type = other RNA
nttgaagtatgcctcaagg